European Patent Specification EP 3 727 588 B1, published August 23, 2023. Title: ADAM10 enzyme activator peptides and related uses for treating diseases characterized by an increase fo the beta amyloid peptide. Applicant: Università degli Studi di Milano. The sequence listing filed with the application follows.

SEQUENCE LISTING (8 sequences)

SEQ ID NO: 1 - protein, 24 aa, ARTIFICIAL SEQUENCE
  ADAM10 activator peptide PEP3
  peptide (1)..(24): ACTIVATOR PEPTIDE
YGRKKRRQRRRGGSGQPPRQRPRG

SEQ ID NO: 2 - protein, 24 aa, ARTIFICIAL SEQUENCE
  ADAM10 activator peptide PEP2
  peptide (1)..(24): ACTIVATOR PEPTIDE
YGRKKRRQRRRGGSGLPPRQRPRL

SEQ ID NO: 3 - protein, 24 aa, ARTIFICIAL SEQUENCE
  ADAM10 activator peptide PEP1
  PEPTIDE (1)..(24): ACTIVATOR PEPTIDE
YGRKKRRQRRRGGSGQPPRQRPRE

SEQ ID NO: 4 - DNA, 72 bp, ARTIFICIAL SEQUENCE
  Nucleotide sequence encoding peptide PEP3
tatggtcgtaagaagcgccgccaacgacgtcgaggcggcagcggacagccccctcgtcagcgcccgcggggt

SEQ ID NO: 5 - protein, 24 aa, ARTIFICIAL SEQUENCE
  Control peptide inPEP3
YGRKKRRQRRRGGSGQPPEQEPRG

SEQ ID NO: 6 - protein, 24 aa, ARTIFICIAL SEQUENCE
  CONTROL PEPTIDE inPEP2
YGRKKRRQRRRGGSGLPPEQEPRL

SEQ ID NO: 7 - protein, 24 aa, ARTIFICIAL SEQUENCE
  CONTROL PEPTIDE inPEP1
YGRKKRRQRRRGGSGQPPEQEPRE

SEQ ID NO: 8 - DNA, 72 bp, ARTIFICIAL SEQUENCE
  Nucleotide sequence encoding for the peptide PEP2
tatggtcgtaagaagcgccgccaacgacgtcgaggcggcagcggacttccccctcgtcaacgccctcgtctc